European Patent Specification EP 3 991 721 B1, published March 4, 2026. Title: Pharmaceutical formulation of Inactivated Polypeptide TRP. Applicant: MET Life Science. The sequence listing filed with the application follows.

SEQUENCE LISTING (29 sequences)

SEQ ID NO: 1 - protein, 114 aa, Homo sapiens
QAKHKQRKRLKSSCKRHPLYVDFSDVGWNDWIVAPPGYHAFYCHGECPFPLADHLNSTNHAIVQTLVNSVNSKIPKACCVPTELSAISMLYLDENEKVVLKNYQDMVVEGCGCR

SEQ ID NO: 2 - protein, 183 aa, Homo sapiens
STGVLLPLQNNELPGAEYQYKKDEVWEERKPYKTLQAQAPEKSKNKKKQRKGPHRKSQTLQFDEQTLKKARRKQWIEPRNCARRYLKVDFADIGWSEWIISPKSFDAYYCSGACQFPMPKSLKPSNHATIQSIVRAVGVVPGIPEPCCVPEKMSSLSILFFDENKNVVLKVYPNMTVESCACR

SEQ ID NO: 3 - protein, 116 aa, Homo sapiens
SPKHHSQRARKKNKNCRRHSLYVDFSDVGWNDWIVAPPGYQAFYCHGDCPFPLADHLNSTNHAIVQTLVNSVNSSIPKACCVPTELSAISMLYLDEYDKVVLKNYQEMVVEGCGCR

SEQ ID NO: 4 - protein, 138 aa, Homo sapiens
AANKRKNQNRNKSSSHQDSSRMSSVGDYNTSEQKQACKKHELYVSFRDLGWQDWIIAPEGYAAFYCDGECSFPLNAHMNATNHAIVQTLVHLMFPDHVPKPCCAPTKLNAISVLYFDDSSNVILKKYRNMVVRSCGCH

SEQ ID NO: 5 - protein, 139 aa, Homo sapiens
SASSRRRQQSRNRSTQSQDVARVSSASDYNSSELKTACRKHELYVSFQDLGWQDWIIAPKGYAANYCDGECSFPLNAHMNATNHAIVQTLVHLMNPEYVPKPCCAPTKLNAISVLYFDDNSNVILKKYRNMVVRACGCH

SEQ ID NO: 6 - protein, 139 aa, Homo sapiens
STGSKQRSQNRSKTPKNQEALRMANVAENSSSDQRQACKKHELYVSFRDLGWQDWIIAPEGYAAYYCEGECAFPLNSYMNATNHAIVQTLVHFINPETVPKPCCAPTQLNAISVLYFDDSSNVILKKYRNMVVRACGCH

SEQ ID NO: 7 - protein, 133 aa, Homo sapiens
RRQPKKSNELPQANRLPGIFDDVHGSHGRQVCRRHELYVSFQDLGWLDWVIAPQGYSAYYCEGECSFPLDSCMNATNHAILQSLVHLMMPDAVPKACCAPTKLSATSVLYYDSSNNVILRKHRNMVVKACGCH

SEQ ID NO: 8 - protein, 110 aa, Homo sapiens
SAGAGSHCQKTSLRVNFEDIGWDSWIIAPKEYEAYECKGGCFFPLADDVTPTKHAIVQTLVHLKFPTKVGKACCVPTKLSPISVLYKDDMGVPTLKYHYEGMSVAECGCR

SEQ ID NO: 9 - protein, 108 aa, Homo sapiens
NAKGNYCKRTPLYIDFKEIGWDSWIIAPPGYEAYECRGVCNYPLAEHLTPTKHAIIQALVHLKNSQKASKACCVPTKLEPISILYLDKGVVTYKFKYEGMAVSECGCR

SEQ ID NO: 10 - protein, 108 aa, Homo sapiens; identical to SEQ ID NO: 9

SEQ ID NO: 11 - protein, 104 aa, Homo sapiens
SRCSRKPLHVDFKELGWDDWIIAPLDYEAYHCEGLCDFPLRSHLEPTNHAIIQTLLNSMAPDAAPASCCVPARLSPISILYIDAANNVVYKQYEDMVVEACGCR

SEQ ID NO: 12 - protein, 120 aa, Homo sapiens
TAFASRHGKRHGKKSRLRCSKKPLHVNFKELGWDDWIIAPLEYEAYHCEGVCDFPLRSHLEPTNHAIIQTLMNSMDPGSTPPSCCVPTKLTPISILYIDAGNNVVYKQYEDMVVESCGCR

SEQ ID NO: 13 - protein, 120 aa, Homo sapiens
APLATRQGKRPSKNLKARCSRKALHVNFKDMGWDDWIIAPLEYEAFHCEGLCEFPLRSHLEPTNHAVIQTLMNSMDPESTPPTCCVPTRLSPISILFIDSANNVVYKQYEDMVVESCGCR

SEQ ID NO: 14 - protein, 281 aa, Homo sapiens
MVAGTRCLLALLLPQVLLGGAAGLVPELGRRKFAAASSGRPSSQPSDEVLSEFELRLLSMFGLKQRPTPSRDAVVPPYMLDLYRRHSGQPGSPAPDHRLERAASRANTVRSFHHEESLEELPETSGKTTRRFFFNLSSIPTEEFITSAELQVFREQMQDALGNNSSFHHRINIYEIIKPATANSKFPVTRLLDTRLVNQNASRWESFDVTPAVMRWTAGHANHGFVVEVAHLEEKQGVSKRHVRISRSLHQDEHSWSQIRPLLVTFGHDGKGHPLHKREKR

SEQ ID NO: 15 - protein, 289 aa, Homo sapiens
MAGASRLLFLWLGCFCVSLAQGERPKPPFPELRKAVPGDRTAGGGPDSELQPQDKVSEHMLRLYDRYSTVQAARTPGSLEGGSQPWRPRLLREGNTVRSFRAAAAETLERKGLYIFNLTSLTKSENILSATLYFCIGELGNISLSCPVSGGCSHHAQRKHIQIDLSAWTLKFSRNQSQLLGHLSVDMAKSHRDIMSWLSKDITQFLRKAKENEEFLIGFNITSKGRQLPKRRLPFPEPYILVYANDAAISEPESVVSSLQGHRNFPTGTVPKWDSHIRAALSIERRKKR

SEQ ID NO: 16 - protein, 292 aa, Homo sapiens
MIPGNRMLMVVLLCQVLLGGASHASLIPETGKKKVAEIQGHAGGRRSGQSHELLRDFEATLLQMFGLRRRPQPSKSAVIPDYMRDLYRLQSGEEEEEQIHSTGLEYPERPASRANTVRSFHHEEHLENIPGTSENSAFRFLFNLSSIPENEAISSAELRLFREQVDQGPDWERGFHRINIYEVMKPPAEVVPGHLITRLLDTRLVHHNVTRWETFDVSPAVLRWTREKQPNYGLAIEVTHLHQTRTHQGQHVRISRSLPQGSGNWAQLRPLLVTFGHDGRGHALTRRRRAKR

SEQ ID NO: 17 - protein, 316 aa, Homo sapiens
MHLTVFLLKGIVGFLWSCWVLVGYAKGGLGDNHVHSSFIYRRLRNHERREIQREILSILGLPHRPRPFSPGKQASSAPLFMLDLYNAMTNEENPEESEYSVRASLAEETRGARKGYPASPNGYPRRIQLSRTTPLTTQSPPLASLHDTNFLNDADMVMSFVNLVERDKDFSHQRRHYKEFRFDLTQIPHGEAVTAAEFRIYKDRSNNRFENETIKISIYQIIKEYTNRDADLFLLDTRKAQALDVGWLVFDITVTSNHWVINPQNNLGLQLCAETGDGRSINVKSAGLVGRQGPQSKQPFMVAFFKASEVLLRSVR

SEQ ID NO: 18 - protein, 374 aa, Homo sapiens
MPGLGRRAQWLCWWWGLLCSCCGPPPLRPPLPAAAAAAAGGQLLGDGGSPGRTEQPPPSPQSSSGFLYRRLKTQEKREMQKEILSVLGLPHRPRPLHGLQQPQPPALRQQEEQQQQQQLPRGEPPPGRLKSAPLFMLDLYNALSADNDEDGASEGERQQSWPHEAASSSQRRQPPPGAAHPLNRKSLLAPGSGSGGASPLTSAQDSAFLNDADMVMSFVNLVEYDKEFSPRQRHHKEFKFNLSQIPEGEVVTAAEFRIYKDCVMGSFKNQTFLISIYQVLQEHQHRDSDLFLLDTRVVWASEEGWLEFDITATSNLWVVTPQHNMGLQLSVVTRDGVHVHPRAAGLVGRDGPYDKQPFMVAFFKVSEVHVRTTR

SEQ ID NO: 19 - protein, 292 aa, Homo sapiens
MHVRSLRAAAPHSFVALWAPLFLLRSALADFSLDNEVHSSFIHRRLRSQERREMQREILSILGLPHRPRPHLQGKHNSAPMFMLDLYNAMAVEEGGGPGGQGFSYPYKAVFSTQGPPLASLQDSHFLTDADMVMSFVNLVEHDKEFFHPRYHHREFRFDLSKIPEGEAVTAAEFRIYKDYIRERFDNETFRISVYQVLQEHLGRESDLFLLDSRTLWASEEGWLVFDITATSNHWVVNPRHNLGLQLSVETLDGQSINPKLAGLIGRHGPQNKQPFMVAFFKATEVHFRSIR

SEQ ID NO: 20 - protein, 269 aa, Homo sapiens
MTALPGPLWLLGLALCALGGGGPGLRPPPGCPQRRLGARERRDVQREILAVLGLPGRPRPRAPPAASRLPASAPLFMLDLYHAMAGDDDEDGAPAERRLGRADLVMSFVNMVERDRALGHQEPHWKEFRFDLTQIPAGEAVTAAEFRIYKVPSIHLLNRTLHVSMFQVVQEQSNRESDLFFLDLQTLRAGDEGWLVLDVTAASDCWLLKRHKDLGLRLYVETEDGHSVDPGLAGLLGQRAPRSQQPFVVTFFRASPSPIRTPRAVRPLR

SEQ ID NO: 21 - protein, 318 aa, Homo sapiens
MCPGALWVALPLLSLLAGSLQGKPLQSWGRGSAGGNAHSPLGVPGGGLPEHTFNLKMFLENVKVDFLRSLNLSGVPSQDKTRVEPPQYMIDLYNRYTSDKSTPASNIVRSFSMEDAISITATEDFPFQKHILLFNISIPRHEQITRAELRLYVSCQNHVDPSHDLKGSVVIYDVLDGTDAWDSATETKTFLVSQDIQDEGWETLEVSSAVKRWVRSDSTKSKNKLEVTVESHRKGCDTLDISVPPGSRNLPFFVVFSNDHSSGTKETRLELREMISHEQESVLKKLSKDGSTEAGESSHEEDTDGHVAAGSTLARRKR

SEQ ID NO: 22 - protein, 316 aa, Homo sapiens
MGSLVLTLCALFCLAAYLVSGSPIMNLEQSPLEEDMSLFGDVFSEQDGVDFNTLLQSMKDEFLKTLNLSDIPTQDSAKVDPPEYMLELYNKFATDRTSMPSANIIRSFKNEDLFSQPVSFNGLRKYPLLFNVSIPHHEEVIMAELRLYTLVQRDRMIYDGVDRKITIFEVLESKGDNEGERNMLVLVSGEIYGTNSEWETFDVTDAIRRWQKSGSSTHQLEVHIESKHDEAEDASSGRLEIDTSAQNKHNPLLIVFSDDQSSDKERKEELNEMISHEQLPELDNLGLDSFSSGPGEEALLQMRSNIIYDSTARIRR

SEQ ID NO: 23 - protein, 316 aa, Homo sapiens; identical to SEQ ID NO: 22

SEQ ID NO: 24 - protein, 346 aa, Homo sapiens
MDLSAAAALCLWLLSACRPRDGLEAAAVLRAAGAGPVRSPGGGGGGGGGGRTLAQAAGAAAVPAAAVPRARAARRAAGSGFRNGSVVPHHFMMSLYRSLAGRAPAGAAAVSASGHGRADTITGFTDQATQDESAAETGQSFLFDVSSLNDADEVVGAELRVLRRGSPESGPGSWTSPPLLLLSTCPGAARAPRLLYSRAAEPLVGQRWEAFDVADAMRRHRREPRPPRAFCLLLRAVAGPVPSPLALRRLGFGWPGGGGSAAEERAVLVVSSRTQRKESLFREIRAQARALGAALASEPLPDPGTGTASPRAVIGGRRRRRTALAGTRTAQGSGGGAGRGHGRRGR

SEQ ID NO: 25 - protein, 335 aa, Homo sapiens
MDTPRVLLSAVFLISFLWDLPGFQQASISSSSSSAELGSTKGMRSRKEGKMQRAPRDSDAGREGQEPQPRPQDEPRAQQPRAQEPPGRGPRVVPHEYMLSIYRTYSIAEKLGINASFFQSSKSANTITSFVDRGLDDLSHTPLRRQKYLFDVSMLSDKEELVGAELRLFRQAPSAPWGPPAGPLHVQLFPCLSPLLLDARTLDPQGAPPAGWEVFDVWQGLRHQPWKQLCLELRAAWGELDAGEAEARARGPQQPPPPDLRSLGFGRRVRPPQERALLVVFTRSQRKNLFAEMREQLGSAEAAGPGAGAEGSWPPPSGAPDARPWLPSPGRRRRR

SEQ ID NO: 26 - protein, 381 aa, Homo sapiens
MRLPKLLTFLLWYLAWLDLEFICTVLGAPDLGQRPQGTRPGLAKAEAKERPPLARNVFRPGGHSYGGGATNANARAKGGTGQTGGLTQPKKDEPKKLPPRPGGPEPKPGHPPQTRQATARTVTPKGQLPGGKAPPKAGSVPSSFLLKKAREPGPPREPKEPFRPPPITPHEYMLSLYRTLSDADRKGGNSSVKLEAGLANTITSFIDKGQDDRGPVVRKQRYVFDISALEKDGLLGAELRILRKKPSDTAKPAAPGGGRAAQLKLSSCPSGRQPASLLDVRSVPGLDGSGWEVFDIWKLFRNFKNSAQLCLELEAWERGRAVDLRGLGFDRAARQVHEKALFLVFGRTKKRDLFFNEIKARSGQDDKTVYEYLFSQRRKRR

SEQ ID NO: 27 - protein, 11 aa, Artificial Sequence
  PTD
YGRKKRRQRRR

SEQ ID NO: 28 - protein, 519 aa, Artificial Sequence
  TRP2
MRGSHHHHHHGMASMTGGQQMGRDLYDDDDKDRWGSKLGYGRKKRRQRRRGGLFGAIAGFIENGWEGMIDGGSTMAGTMHVRSLRAAAPHSFVALWAPLFLLRSALADFSLDNEVHSSFIHRRLRSQERREMQREILSILGLPHRPRPHLQGKHNSAPMFMLDLYNAMAVEEGGGPGGQGFSYPYKAVFSTQGPPLASLQDSHFLTDADMVMSFVNLVEHDKEFFHPRYHHREFRFDLSKIPEGEAVTAAEFRIYKDYIRERFDNETFRISVYQVLQEHLGRESDLFLLDSRTLWASEEGWLVFDITATSNHWVVNPRHNLGLQLSVETLDGQSINPKLAGLIGRHGPQNKQPFMVAFFKATEVHFRSIRSTGSKQRSQNRSKTPKNQEALRMANVAENSSSDQRQACKKHELYVSFRDLGWQDWIIAPEGYAAYYCEGECAFPLNSYMNATNHAIVQTLVHFINPETVPKPCCAPTQLNAISVLYFDDSSNVILKKYRNMVVRACGCHHYPYDVPDYA

SEQ ID NO: 29 - DNA, 1353 bp, Artificial Sequence
  mCherry-Rab7a vector
atggtgagcaagggcgaggaggataacatggccatcatcaaggagttcatgcgcttcaaggtgcacatggagggctccgtgaacggccacgagttcgagatcgagggcgagggcgagggccgcccctacgagggcacccagaccgccaagctgaaggtgaccaagggtggccccctgcccttcgcctgggacatcctgtcccctcagttcatgtacggctccaaggcctacgtgaagcaccccgccgacatccccgactacttgaagctgtccttccccgagggcttcaagtgggagcgcgtgatgaacttcgaggacggcggcgtggtgaccgtgacccaggactcctccctgcaggacggcgagttcatctacaaggtgaagctgcgcggcaccaacttcccctccgacggccccgtaatgcagaagaagaccatgggctgggaggcctcctccgagcggatgtaccccgaggacggcgccctgaagggcgagatcaagcagaggctgaagctgaaggacggcggccactacgacgctgaggtcaagaccacctacaaggccaagaagcccgtgcagctgcccggcgcctacaacgtcaacatcaagttggacatcacctcccacaacgaggactacaccatcgtggaacagtacgaacgcgccgagggccgccactccaccggcggcatggacgagctgtacaagggaggtaagggtaaaggtggtatgacctctaggaagaaagtgttgctgaaggttatcatcctgggagattctggagtcgggaagacatcactcatgaaccagtatgtgaataagaaattcagcaatcagtacaaagccacaataggagctgactttctgaccaaggaggtgatggtggatgacaggctagtcacaatgcagatatgggacacagcaggacaggaacggttccagtctctcggtgtggccttctacagaggtgcagactgctgcgttctggtatttgatgtgactgcccccaacacattcaaaaccctagatagctggagagatgagtttctcatccaggccagtccccgagatcctgaaaacttcccatttgttgtgttgggaaacaagattgacctcgaaaacagacaagtggccacaaagcgggcacaggcctggtgctacagcaaaaacaacattccctactttgagaccagtgccaaggaggccatcaacgtggagcaggcgttccagacgattgcacggaatgcacttaagcaggaaacggaggtggagctgtacaacgaatttcctgaacctatcaaactggacaagaatgaccgggccaaggcctcggcagaaagctgcagttgctga